European Patent Specification EP 3 896 156 B1, published July 17, 2024. Title: Recombinant Hydrogenophilus bacterium having improved valine-producing ability. Applicant: Utilization of Carbon Dioxide Institute Co., Ltd. The sequence listing filed with the application follows.

SEQUENCE LISTING (14 sequences)

SEQ ID NO: 1 - protein, 163 aa, Hydrogenophilus thermoluteolus
MRHVIALLVENESGALSRIAGLFSARGYNIESLTVAPTEDESLSRMTIVTTGSDDVIEQITKQLNKLIDTVKVVDLSESAHIERELMMVKVRAVGSDREELKRLADIFRARIIDVTDTTYVIELTGNQQKLNAFLAAISPSLILETVRSGVCGIARGERMLKA

SEQ ID NO: 2 - DNA, 492 bp, Hydrogenophilus thermoluteolus
atgagacacgtgattgcactgctggtggaaaacgaatcgggcgcgttgtcgcgcatcgccgggctcttttcggcgcgtggctacaacatcgaatcgctcaccgtcgcaccgaccgaagacgagagcctgtcgcggatgacgatcgtcaccaccggttcggacgacgtgatcgaacagatcaccaagcagctcaacaaactgatcgatacggtcaaagtggtcgacctctccgaatccgcgcacatcgagcgcgaactgatgatggtgaaggtccgtgccgtgggatcagaccgcgaagagctcaaacgcctggccgacatcttccgcgcccggatcatcgacgtcaccgacaccacctacgtgatcgaactcaccggcaaccagcagaagctcaacgcgtttctggcggcgatctcgcccagtctcatcttggagacggtgcgtagcggcgtctgcggcattgcccgtggcgagcgtatgttgaaagcctga

SEQ ID NO: 3 - DNA, 396 bp, Hydrogenophilus thermoluteolus
atgccaaccatcaaccagttggtgcgtcgtccgcggaaaacggcgcccgaaaagagcaaagtgccggcgttgcagggatgtccgcaaaaacgaggcgtgtgtacgcgcgtctataccacgacgccgaaaaagccgaactcggcccttcgtaaggtcgcgaaagtgcgtttgaccaacggttacgaggtgatttcgtacatcggcggcgaagggcacaatctgcaagaacactcggtggtgctgattcgtggcggccgggtgaaagacctgccgggtgtgcgttaccacatcgtgcgcggttcgctcgacttgcaaggggtcaaggaccgtaagcaagggcgttccaagtacggggcgaagcgtccgaagccgggcgccgctgcgggcaagaaataa

SEQ ID NO: 4 - DNA, 1026 bp, Escherichia coli
atgaaaaagcctgaactcaccgcgacatctgtcgagaagtttctgatcgaaaagttcgacagcgtctccgacctgatgcagctctcggagggcgaagaatctcgtgctttcagcttcgatgtaggagggcgtggatatgtcctgcgggtaaatagctgcgccgatggtttctacaaagatcgttatgtttatcggcactttgcatcggccgcgctcccgattccggaagtgcttgacattggggaattcagcgagagcctgacctattgcatctcccgccgtgcacagggtgtcacgttgcaagacctgcctgaaaccgaactgcccgctgttctgcagccggtcgcggaggccatggatgcgatcgctgcggccgatcttagccagacgagcgggttcggcccattcggaccgcaaggaatcggtcaatacactacatggcgtgatttcatatgcgcgattgctgatccccatgtgtatcactggcaaactgtgatggacgacaccgtcagtgcgtccgtcgcgcaggctctcgatgagctgatgctttgggccgaggactgccccgaagtccggcacctcgtgcacgcggatttcggctccaacaatgtcctgacggacaatggccgcataacagcggtcattgactggagcgaggcgatgttcggggattcccaatacgaggtcgccaacatcttcttctggaggccgtggttggcttgtatggagcagcagacgcgctacttcgagcggaggcatccggagcttgcaggatcgccgcggctccgggcgtatatgctccgcattggtcttgaccaactctatcagagcttggttgacggcaatttcgatgatgcagcttgggcgcagggtcgatgcgacgcaatcgtccgatccggagccgggactgtcgggcgtacacaaatcgcccgcagaagcgcggccgtctggaccgatggctgtgtagaagtactcgccgatagtggaaaccgacgccccagcactcgtccgagggcaaaggaatag

SEQ ID NO: 5 - DNA, 795 bp, Escherichia coli
atgattgaacaagatggattgcacgcaggttctccggccgcttgggtggagaggctattcggctatgactgggcacaacagacaatcggctgctctgatgccgccgtgttccggctgtcagcgcaggggcgcccggttctttttgtcaagaccgacctgtccggtgccctgaatgaactccaagacgaggcagcgcggctatcgtggctggccacgacgggcgttccttgcgcagctgtgctcgacgttgtcactgaagcgggaagggactggctgctattgggcgaagtgccggggcaggatctcctgtcatctcaccttgctcctgccgagaaagtatccatcatggctgatgcaatgcggcggctgcatacgcttgatccggctacctgcccattcgaccaccaagcgaaacatcgcatcgagcgagcacgtactcggatggaagccggtcttgtcgatcaggatgatctggacgaagagcatcaggggctcgcgccagccgaactgttcgccaggctcaaggcgcggatgcccgacggcgaggatctcgtcgtgacccatggcgatgcctgcttgccgaatatcatggtggaaaatggccgcttttctggattcatcgactgtggccggctgggtgtggcggaccgctatcaggacatagcgttggctacccgtgatattgctgaagagcttggcggcgaatgggctgaccgcttcctcgtgctttacggtatcgccgctcccgattcgcagcgcatcgccttctatcgccttcttgacgagttcttctga

SEQ ID NO: 6 - DNA, 762 bp, Staphylococcus aureus
atgaatggaccaataataatgactagagaagaaagaatgaagattgttcatgaaattaaggaacgaatattggataaatatggggatgatgttaaggctattggtgtttatggctctcttggtcgtcagactgatgggccctattcggatattgagatgatgtgtgtcatgtcaacagaggaagcagagttcagccatgaatggacaaccggtgagtggaaggtggaagtgaattttgatagcgaagagattctactagattatgcatctcaggtggaatcagattggccgcttacacatggtcaatttttctctattttgccgatttatgattcaggtggatacttagagaaagtgtatcaaactgctaaatcggtagaagcccaaacgttccacgatgcgatttgtgcccttatcgtagaagagctgtttgaatatgcaggcaaatggcgtaatattcgtgtgcaaggaccgacaacatttctaccatccttgactgtacaggtagcaatggcaggtgccatgttgattggtctgcatcatcgcatctgttatacgacgagcgcttcggtcttaactgaagcagttaagcaatcagatcttccttcaggttatgaccatctgtgccagttcgtaatgtctggtcaactttccgactctgagaaacttctggaatcgctagagaatttctggaatgggattcaggagtggacagaacgacacggatatatagtggatgtgtcaaaacgcataccattttga

SEQ ID NO: 7 - DNA, 35 bp, Artificial sequence
  PCR primer
atacgcgtcctccgatgcgtcgtaagggaaacgtc

SEQ ID NO: 8 - DNA, 35 bp, Artificial sequence
  PCR primer
atagtcgacttatttcttgcccgcagcggcgcccg

SEQ ID NO: 9 - DNA, 35 bp, Artificial sequence
  PCR primer
atactcgaggagatgacgttggaggggcaaggtcg

SEQ ID NO: 10 - DNA, 35 bp, Artificial sequence
  PCR primer
atacgcgtctattcctttgccctcggacgagtgct

SEQ ID NO: 11 - DNA, 35 bp, Artificial sequence
  PCR primer
atgaattccccggaagcgacaagcagttcctgggg

SEQ ID NO: 12 - DNA, 35 bp, Artificial sequence
  PCR primer
acaacgcgtccgattcgttttccaccagcagtgca

SEQ ID NO: 13 - DNA, 35 bp, Artificial sequence
  PCR primer
cggacgcgttgtcgcgcatcgccgggctcttttcg

SEQ ID NO: 14 - DNA, 35 bp, Artificial sequence
  PCR primer
ttctgcaggcgctttgccgctttggtcctgatgca